European Patent Application EP 4 585 691 A1, published July 16, 2025. Title: Construct of self-circularization RNA. Applicant: Rznomics Inc. Application KR. The sequence listing filed with the application follows.

SEQUENCE LISTING (98 sequences)

SEQ ID NO: 1-2 - skipped (2 entries)

SEQ ID NO: 3 - DNA, 20 bp, synthetic construct
  misc_feature 1..20: note = T7 promoter
  source 1..20: mol_type = other DNA
taatacgactcactataggg

SEQ ID NO: 4 - DNA, 151 bp, synthetic construct
  misc_feature 1..151: note = AS 150
  source 1..151: mol_type = other DNA
cggcggccagcatggagaactgccatggctcagccaggtagtactgtgggtactcgaagtggctgcgtaccacacccgtcgcattggagaagggcacgtagaagttagggccttctgtgccattcatggctgtggcccttgtggctgaccc

SEQ ID NO: 5 - skipped

SEQ ID NO: 6 - DNA, 387 bp, synthetic construct
  misc_feature 1..387: note = Trans splicing ribozyme
  source 1..387: mol_type = other DNA
aaaagttatcaggcatgcacctggtagctagtctttaaaccaatagattgcatcggtttaaaaggcaagaccgtcaaattgcgggaaaggggtcaacagccgttcagtaccaagtctcaggggaaactttgagatggccttgcaaagggtatggtaataagctgacggacatggtcctaaccacgcagccaagtcctaagtcaacagatcttctgttgatatggatgcagttcacagactaaatgtcggtcggggaagatgtattcttctcataagatatagtcggacctctccttaatgggagctagcggatgaagtgatgcaacactggagccgctgggaactaatttgtatgcgaaagtatattgattagttttggagtactcg

SEQ ID NO: 7 - DNA, 463 bp, synthetic construct
  misc_feature 1..463: note = EMCV IRES
  source 1..463: mol_type = other DNA
gagggcccggaaacctggccctgtcttcttgacgagcattcctaggggtctttcccctctcgccaaaggaatgcaaggtctgttgaatgtcgtgaaggaagcagttcctctggaagcttcttgaagacaaacaacgtctgtagcgaccctttgcaggcagcggaaccccccacctggcgacaggtgcctctgcggccaaaagccacgtgtataagatacacctgcaaaggcggcacaaccccagtgccacgttgtgagttggatagttgtggaaagagtcaaatggctctcctcaagcgtattcaacaaggggctgaaggatgcccagaaggtaccccattgtatgggatctgatctggggcctcggtgcacatgctttacatgtgtttagtcgaggttaaaaaaacgtctaggccccccgaaccacggggacgtggttttcctttgaaaaacacgatgataa

SEQ ID NO: 8 - DNA, 558 bp, synthetic construct
  misc_feature 1..558: note = Gaussia Luciferase
  source 1..558: mol_type = other DNA
atgggagtcaaagttctgtttgccctgatctgcatcgctgtggccgaggccaagcccaccgagaacaacgaagacttcaacatcgtggccgtggccagcaacttcgcgaccacggatctcgatgctgaccgcgggaagttgcccggcaagaagctgccgctggaggtgctcaaagagatggaagccaatgcccggaaagctggctgcaccaggggctgtctgatctgcctgtcccacatcaagtgcacgcccaagatgaagaagttcatcccaggacgctgccacacctacgaaggcgacaaagagtccgcacagggcggcataggcgaggcgatcgtcgacattcctgagattcctgggttcaaggacttggagcccatggagcagttcatcgcacaggtcgatctgtgtgtggactgcacaactggctgcctcaaagggcttgccaacgtgcagtgttctgacctgctcaagaagtggctgccgcaacgctgtgcgacctttgccagcaagatccagggccaggtggacaagatcaagggggccggtggtgactaa

SEQ ID NO: 9 - DNA, 150 bp, synthetic construct
  misc_feature 1..150: note = Antisense Binding Sequecne
  source 1..150: mol_type = other DNA
gggtcagccacaagggccacagccatgaatggcacagaaggccctaacttctacgtgcccttctccaatgcgacgggtgtggtacgcagccacttcgagtacccacagtactacctggctgagccatggcagttctccatgctggccgcc

SEQ ID NO: 10 - DNA, 1908 bp, synthetic construct
  misc_feature 1..1908: note = DNA template encoding self-circularizaion RNA of the example 1
  source 1..1908: mol_type = other DNA
gggattcgaacatcgattaatacgactcactataggggcatcgattgaattgtcgacgaattcggcggccagcatggagaactgccatggctcagccaggtagtactgtgggtactcgaagtggctgcgtaccacacccgtcgcattggagaagggcacgtagaagttagggccttctgtgccattcatggctgtggcccttgtggctgacccgaattccgtactccgcccaaaaaagttatcaggcatgcacctggtagctagtctttaaaccaatagattgcatcggtttaaaaggcaagaccgtcaaattgcgggaaaggggtcaacagccgttcagtaccaagtctcaggggaaactttgagatggccttgcaaagggtatggtaataagctgacggacatggtcctaaccacgcagccaagtcctaagtcaacagatcttctgttgatatggatgcagttcacagactaaatgtcggtcggggaagatgtattcttctcataagatatagtcggacctctccttaatgggagctagcggatgaagtgatgcaacactggagccgctgggaactaatttgtatgcgaaagtatattgattagttttggagtactcgcgagtacgcttaagaaaaaaaaaagagggcccggaaacctggccctgtcttcttgacgagcattcctaggggtctttcccctctcgccaaaggaatgcaaggtctgttgaatgtcgtgaaggaagcagttcctctggaagcttcttgaagacaaacaacgtctgtagcgaccctttgcaggcagcggaaccccccacctggcgacaggtgcctctgcggccaaaagccacgtgtataagatacacctgcaaaggcggcacaaccccagtgccacgttgtgagttggatagttgtggaaagagtcaaatggctctcctcaagcgtattcaacaaggggctgaaggatgcccagaaggtaccccattgtatgggatctgatctggggcctcggtgcacatgctttacatgtgtttagtcgaggttaaaaaaacgtctaggccccccgaaccacggggacgtggttttcctttgaaaaacacgatgataagcttgccacaacccttaagaccggtatgggagtcaaagttctgtttgccctgatctgcatcgctgtggccgaggccaagcccaccgagaacaacgaagacttcaacatcgtggccgtggccagcaacttcgcgaccacggatctcgatgctgaccgcgggaagttgcccggcaagaagctgccgctggaggtgctcaaagagatggaagccaatgcccggaaagctggctgcaccaggggctgtctgatctgcctgtcccacatcaagtgcacgcccaagatgaagaagttcatcccaggacgctgccacacctacgaaggcgacaaagagtccgcacagggcggcataggcgaggcgatcgtcgacattcctgagattcctgggttcaaggacttggagcccatggagcagttcatcgcacaggtcgatctgtgtgtggactgcacaactggctgcctcaaagggcttgccaacgtgcagtgttctgacctgctcaagaagtggctgccgcaacgctgtgcgacctttgccagcaagatccagggccaggtggacaagatcaagggggccggtggtgactaaaaaaaaaaaaaccggtttgggtgggagcagccacgggtcagccacaagggccacagccatgaatggcacagaaggccctaacttctacgtgcccttctccaatgcgacgggtgtggtacgcagccacttcgagtacccacagtactacctggctgagccatggcagttctccatgctggccgccaagcttgcctcgagcagcgctgctcgagagatct

SEQ ID NO: 11 - DNA, 56 bp, synthetic construct
  misc_feature 1..56: note = T7 Circular Forward primer
  source 1..56: mol_type = other DNA
gggattcgaacatcgattaatacgactcactataggggcatcgattgaattgtcga

SEQ ID NO: 12 - DNA, 34 bp, synthetic construct
  misc_feature 1..34: note = T7 Circular Reverse primer
  source 1..34: mol_type = other DNA
agatctctcgagcagcgctgctcgaggcaagctt

SEQ ID NO: 13 - DNA, 21 bp, synthetic construct
  misc_feature 1..21: note = Circular STS Forward primer of the example 2-2
  source 1..21: mol_type = other DNA
ccctgagtggctgagctcagg

SEQ ID NO: 14 - DNA, 23 bp, synthetic construct
  misc_feature 1..23: note = Circular STS Reverse primer of the example 2-2
  source 1..23: mol_type = other DNA
cagcaagcatactaaattgccag

SEQ ID NO: 15 - DNA, 25 bp, synthetic construct
  misc_feature 1..25: note = Circular STS Forward primer of the example 3
  source 1..25: mol_type = other DNA
caaggacttggagcccatggagcag

SEQ ID NO: 16 - DNA, 23 bp, synthetic construct
  misc_feature 1..23: note = Circular STS Reverse primer 2 of the example 3
  source 1..23: mol_type = other DNA
tgtgccgcctttgcaggtgtatc

SEQ ID NO: 17 - DNA, 50 bp, synthetic construct
  misc_feature 1..50: note = AS50
  source 1..50: mol_type = other DNA
aagttagggccttctgtgccattcatggctgtggcccttgtggctgaccc

SEQ ID NO: 18 - DNA, 100 bp, synthetic construct
  misc_feature 1..100: note = AS100
  source 1..100: mol_type = other DNA
actcgaagtggctgcgtaccacacccgtcgcattggagaagggcacgtagaagttagggccttctgtgccattcatggctgtggcccttgtggctgaccc

SEQ ID NO: 19 - DNA, 150 bp, synthetic construct
  misc_feature 1..150: note = AS150
  source 1..150: mol_type = other DNA
ggcggccagcatggagaactgccatggctcagccaggtagtactgtgggtactcgaagtggctgcgtaccacacccgtcgcattggagaagggcacgtagaagttagggccttctgtgccattcatggctgtggcccttgtggctgaccc

SEQ ID NO: 20 - DNA, 200 bp, synthetic construct
  misc_feature 1..200: note = AS200
  source 1..200: mol_type = other DNA
agcgtgaggaagttgatggggaagcccagcacgatcagcagaaacatgtaggcggccagcatggagaactgccatggctcagccaggtagtactgtgggtactcgaagtggctgcgtaccacacccgtcgcattggagaagggcacgtagaagttagggccttctgtgccattcatggctgtggcccttgtggctgaccc

SEQ ID NO: 21 - DNA, 250 bp, synthetic construct
  misc_feature 1..250: note = AS250
  source 1..250: mol_type = other DNA
ggatgtagttgagaggcgtgcgcagcttcttgtgctggacggtgacgtagagcgtgaggaagttgatggggaagcccagcacgatcagcagaaacatgtaggcggccagcatggagaactgccatggctcagccaggtagtactgtgggtactcgaagtggctgcgtaccacacccgtcgcattggagaagggcacgtagaagttagggccttctgtgccattcatggctgtggcccttgtggctgaccc

SEQ ID NO: 22 - DNA, 300 bp, synthetic construct
  misc_feature 1..300: note = AS300
  source 1..300: mol_type = other DNA
ggtgaagccacctaggaccatgaagaggtcagccacggctaggttgagcaggatgtagttgagaggcgtgcgcagcttcttgtgctggacggtgacgtagagcgtgaggaagttgatggggaagcccagcacgatcagcagaaacatgtaggcggccagcatggagaactgccatggctcagccaggtagtactgtgggtactcgaagtggctgcgtaccacacccgtcgcattggagaagggcacgtagaagttagggccttctgtgccattcatggctgtggcccttgtggctgaccc

SEQ ID NO: 23 - DNA, 10 bp, synthetic construct
  misc_feature 1..10: note = A10
  source 1..10: mol_type = other DNA
aaaaaaaaaa

SEQ ID NO: 24 - DNA, 30 bp, synthetic construct
  misc_feature 1..30: note = A30
  source 1..30: mol_type = other DNA
aaaaaaaaaaaaaaaaaaaaaaaaaaaaaa

SEQ ID NO: 25 - DNA, 39 bp, synthetic construct
  misc_feature 1..39: note = A50
  source 1..39: mol_type = other DNA
aaaaaaaaaaaaaaaaaaaaaaaaaaaaaaaaaaaaaaa

SEQ ID NO: 26 - DNA, 35 bp, synthetic construct
  misc_feature 1..35: note = Control spacer 1
  source 1..35: mol_type = other DNA
ggtagtggtgctactaacttcagcctgctgaagca

SEQ ID NO: 27 - DNA, 34 bp, synthetic construct
  misc_feature 1..34: note = Control spacer 2
  source 1..34: mol_type = other DNA
ggtagtaaactactaactacaacctgctgaagca

SEQ ID NO: 28 - skipped

SEQ ID NO: 29 - DNA, 1522 bp, synthetic construct
  misc_feature 1..1522: note = DNA template encoding self-circularizaion RNA of the example 7
  source 1..1522: mol_type = other DNA
gggattcgaacatcgattaatacgactcactataggggcccaaaaaagttatcaggcatgcacctggtagctagtctttaaaccaatagattgcatcggtttaaaaggcaagaccgtcaaattgcgggaaaggggtcaacagccgttcagtaccaagtctcaggggaaactttgagatggccttgcaaagggtatggtaataagctgacggacatggtcctaaccacgcagccaagtcctaagtcaacagatcttctgttgatatggatgcagttcacagactaaatgtcggtcggggaagatgtattcttctcataagatatagtcggacctctccttaatgggagctagcggatgaagtgatgcaacactggagccgctgggaactaatttgtatgcgaaagtatattgattagttttggagtactcgcgagtacgcttaagaaaaaaaaaagagggcccggaaacctggccctgtcttcttgacgagcattcctaggggtctttcccctctcgccaaaggaatgcaaggtctgttgaatgtcgtgaaggaagcagttcctctggaagcttcttgaagacaaacaacgtctgtagcgaccctttgcaggcagcggaaccccccacctggcgacaggtgcctctgcggccaaaagccacgtgtataagatacacctgcaaaggcggcacaaccccagtgccacgttgtgagttggatagttgtggaaagagtcaaatggctctcctcaagcgtattcaacaaggggctgaaggatgcccagaaggtaccccattgtatgggatctgatctggggcctcggtgcacatgctttacatgtgtttagtcgaggttaaaaaaacgtctaggccccccgaaccacggggacgtggttttcctttgaaaaacacgatgataagcttgccacaacccttaagaccggtatgggagtcaaagttctgtttgccctgatctgcatcgctgtggccgaggccaagcccaccgagaacaacgaagacttcaacatcgtggccgtggccagcaacttcgcgaccacggatctcgatgctgaccgcgggaagttgcccggcaagaagctgccgctggaggtgctcaaagagatggaagccaatgcccggaaagctggctgcaccaggggctgtctgatctgcctgtcccacatcaagtgcacgcccaagatgaagaagttcatcccaggacgctgccacacctacgaaggcgacaaagagtccgcacagggcggcataggcgaggcgatcgtcgacattcctgagattcctgggttcaaggacttggagcccatggagcagttcatcgcacaggtcgatctgtgtgtggactgcacaactggctgcctcaaagggcttgccaacgtgcagtgttctgacctgctcaagaagtggctgccgcaacgctgtgcgacctttgccagcaagatccagggccaggtggacaagatcaagggggccggtggtgactaaaaaaaaaaaaaccggtttgggt

SEQ ID NO: 30-46 - skipped (17 entries)

SEQ ID NO: 47 - RNA, 17 nt, synthetic construct
  misc_feature 1..17: note = Fig 13_P1&P10_5' end
  source 1..17: mol_type = other RNA
gggcgtactccgcccaa

SEQ ID NO: 48 - skipped

SEQ ID NO: 49 - RNA, 17 nt, synthetic construct
  misc_feature 1..17: note = Fig 13_P1&P10+AS150_5' end
  source 1..17: mol_type = other RNA
gggcgtactccgcccaa

SEQ ID NO: 50-89 - skipped (40 entries)

SEQ ID NO: 90 - DNA, 52 bp, synthetic construct
  misc_feature 1..52: note = T7 AU rich #X F primer
  source 1..52: mol_type = other DNA
  variation 23..27: note = n is any one of A, G, C, and T
ataatacgactcactataggggnnnnnaaaagttatcaggcatgcacctggt

SEQ ID NO: 91 - DNA, 35 bp, synthetic construct
  misc_feature 1..35: note = AU rich #X R primer
  source 1..35: mol_type = other DNA
  variation 2..6: note = n is any one of A, G, C, and T
annnnnaccggtttttttttttttagtcaccaccg

SEQ ID NO: 92 - DNA, 1498 bp, synthetic construct
  misc_feature 1..1498: note = Fig. 23c_GOI: CVB3 IRES-sGFP
  source 1..1498: mol_type = other DNA
ttaaaacagcctgtgggttgatcccacccacaggcccattgggcgctagcactctggtatcacggtacctttgtgcgcctgttttataccccctcccccaactgtaacttagaagtaacacacaccgatcaacagtcagcgtggcacaccagccacgttttgatcaagcacttctgttaccccggactgagtatcaatagactgctcacgcggttgaaggagaaagcgttcgttatccggccaactacttcgaaaaacctagtaacaccgtggaagttgcagagtgtttcgctcagcactaccccagtgtagatcaggtcgatgagtcaccgcattccccacgggcgaccgtggcggtggctgcgttggcggcctgcccatggggaaacccatgggacgctctaatacagacatggtgcgaagagtctattgagctagttggtagtcctccggcccctgaatgcggctaatcctaactgcggagcacacaccctcaagccagagggcagtgtgtcgtaacgggcaactctgcagcggaaccgactactttgggtgtccgtgtttcattttattcctatactggctgcttatggtgacaattgagagatcgttaccatatagctattggattggccatccggtgactaatagagctattatatatccctttgttgggtttataccacttagcttgaaagaggttaaaacattacaattcattgttaagttgaatacagcaaaatgcgtaaaggcgaagagctgttcactggtgtcgtccctattctggtggaactggatggtgatgtcaacggtcataagttttccgtgcgtggcgagggtgaaggtgacgcaactaatggtaaactgacgctgaagttcatctgtactactggtaaactgccggtaccttggccgactctggtaacgacgctgacttatggtgttcagtgctttgctcgttatccggaccatatgaagcagcatgacttcttcaagtccgccatgccggaaggctatgtgcaggaacgcacgatttcctttaaggatgacggcacgtacaaaacgcgtgcggaagtgaaatttgaaggcgataccctggtaaaccgcattgagctgaaaggcattgactttaaagaagacggcaatatcctgggccataagctggaatacaattttaacagccacaatgtttacatcaccgccgataaacaaaaaaatggcattaaagcgaattttaaaattcgccacaacgtggaggatggcagcgtgcagctggctgatcactaccagcaaaacactccaatcggtgatggtcctgttctgctgccagacaatcactatctgagcacgcaaagcgttctgtctaaagatccgaacgagaaacgcgatcatatggttctgctggagttcgtaaccgcagcgggcatcacgcatggtatggatgaactgtacaaatgaaaaaaacaaaaaacaaaacaaaaacaaaaaacaaaaaaaa

SEQ ID NO: 93 - DNA, 108 bp, synthetic construct
  misc_feature 1..108: note = AC108 Spacer
  source 1..108: mol_type = other DNA
aaaaaacaaaaaacaaaacggctattatgcgttaccggcgccggaaacgcaatagccgaaaaacaaaaaacaaaaaaaacaaaaaaaaaaccaaaaaaacaaaacaca

SEQ ID NO: 94 - DNA, 1911 bp, synthetic construct
  misc_feature 1..1911: note = Fig. 23d_DNA template for expression of self-circularization RNA comprising recontructed GOI(CVB3 IRES-sGFP)
  source 1..1911: mol_type = other DNA
taatacgactcactataggggataaaaaaagttatcaggcatgcacctggtagctagtctttaaaccaatagattgcatcggtttaaaaggcaagaccgtcaaattgcgggaaaggggtcaacagccgttcagtaccaagtctcaggggaaactttgagatggccttgcaaagggtatggtaataagctgacggacatggtcctaaccacgcagccaagtcctaagtcaacagatcttctgttgatatggatgcagttcacagactaaatgtcggtcggggaagatgtattcttctcataagatatagtcggacctctccttaatgggagctagcggatgaagtgatgcaacactggagccgctgggaactaatttgtatgcgaaagtatattgattagttttggagtactcgcctatactggctgcttatggtgacaattgagagatcgttaccatatagctattggattggccatccggtgactaatagagctattatatatccctttgttgggtttataccacttagcttgaaagaggttaaaacattacaattcattgttaagttgaatacagcaaaatgcgtaaaggcgaagagctgttcactggtgtcgtccctattctggtggaactggatggtgatgtcaacggtcataagttttccgtgcgtggcgagggtgaaggtgacgcaactaatggtaaactgacgctgaagttcatctgtactactggtaaactgccggtaccttggccgactctggtaacgacgctgacttatggtgttcagtgctttgctcgttatccggaccatatgaagcagcatgacttcttcaagtccgccatgccggaaggctatgtgcaggaacgcacgatttcctttaaggatgacggcacgtacaaaacgcgtgcggaagtgaaatttgaaggcgataccctggtaaaccgcattgagctgaaaggcattgactttaaagaagacggcaatatcctgggccataagctggaatacaattttaacagccacaatgtttacatcaccgccgataaacaaaaaaatggcattaaagcgaattttaaaattcgccacaacgtggaggatggcagcgtgcagctggctgatcactaccagcaaaacactccaatcggtgatggtcctgttctgctgccagacaatcactatctgagcacgcaaagcgttctgtctaaagatccgaacgagaaacgcgatcatatggttctgctggagttcgtaaccgcagcgggcatcacgcatggtatggatgaactgtacaaatgaaaaaaacaaaaaacaaaacaaaaacaaaaaacaaaaaaaattaaaacagcctgtgggttgatcccacccacaggcccattgggcgctagcactctggtatcacggtacctttgtgcgcctgttttataccccctcccccaactgtaacttagaagtaacacacaccgatcaacagtcagcgtggcacaccagccacgttttgatcaagcacttctgttaccccggactgagtatcaatagactgctcacgcggttgaaggagaaagcgttcgttatccggccaactacttcgaaaaacctagtaacaccgtggaagttgcagagtgtttcgctcagcactaccccagtgtagatcaggtcgatgagtcaccgcattccccacgggcgaccgtggcggtggctgcgttggcggcctgcccatggggaaacccatgggacgctctaatacagacatggtgcgaagagtctattgagctagttggtagtcctccggcccctgaatgcggctaatcctaactgcggagcacacaccctcaagccagagggcagtgtgtcgtaacgggcaactctgcagcggaaccgactactttgggtgtccgtgtttcattttatt

SEQ ID NO: 95 - DNA, 1717 bp, synthetic construct
  misc_feature 1..1717: note = Fig. 26a_GOI: CVB3 IRES-R.Luciferase mutant
  source 1..1717: mol_type = other DNA
ttaaaacagcctgtgggttgatcccacccacaggcccattgggcgctagcactctggtatcacggtacctttgtgcgcctgttttataccccctcccccaactgtaacttagaagtaacacacaccgatcaacagtcagcgtggcacaccagccacgttttgatcaagcacttctgttaccccggactgagtatcaatagactgctcacgcggttgaaggagaaagcgttcgttatccggccaactacttcgaaaaacctagtaacaccgtggaagttgcagagtgtttcgctcagcactaccccagtgtagatcaggtcgatgagtcaccgcattccccacgggcgaccgtggcggtggctgcgttggcggcctgcccatggggaaacccatgggacgctctaatacagacatggtgcgaagagtctattgagctagttggtagtcctccggcccctgaatgcggctaatcctaactgcggagcacacaccctcaagccagagggcagtgtgtcgtaacgggcaactctgcagcggaaccgactactttgggtgtccgtgtttcattttattcctatactggctgcttatggtgacaattgagagatcgttaccatatagctattggattggccatccggtgactaatagagctattatatatccctttgttgggtttataccacttagcttgaaagaggttaaaacattacaattcattgttaagttgaatacagcaaaatggcttccaaggtgtacgaccccgagcaacgcaaacgcatgatcactgggcctcagtggtgggctcgctgcaagcaaatgaacgtgctggactccttcatcaactactatgattccgagaagcacgccgagaacgccgtgatttttctgcatggtaacgctgcctccagctacctgtggaggcacgtcgtgcctcacatcgagcccgtggctagatgcatcatccctgatctgatcggaatgggtaagtccggcaagagcgggaatggctcatatcgcctcctggatcactacaagtacctcaccgcttggttcgagctgctgaaccttccaaagaaaatcatctttgtgggccacgactggggggcttgtctggcctttcactactcctacgagcaccaagacaagatcaaggccatcgtccatgctgagagtgtcgtggacgtgatcgagtcctgggacgagtggcctgacatcgaggaggatatcgccctgatcaagagcgaagagggcgagaaaatggtgcttgagaataacttcttcgtcgagaccgtcctcccaagcaagatcatgcggaaactggagcctgaggagttcgctgcctacctggagccattcaaggagaagggcgaggttagacggcctaccctctcctggcctcgcgagatccctctcgttaagggaggcaagcccgacgtcgtcgcaattgtccgcaactacaacgcctaccttcgggccagcgacgatctgcctaagatgttcatcgagtccgaccctgggttcttttccaacgctattgtcgagggagctaagaagttccctaacaccgagttcgtgaaggtgaagggcctccacttcagccaggaggacgctccagatgaaatgggtaagtacatcaagagcttcgtggagcgcgtgctgaagaacgagcagtaaaaaaaacaaaaaacaaaacaaaaacaaaaaacaaaaaaaa

SEQ ID NO: 96 - DNA, 2130 bp, synthetic construct
  misc_feature 1..2130: note = Fig. 26b_DNA template for expression of self-circularization RNA comprising recontructed GOI(CVB3 IRES-R.Luciferase mutant)
  source 1..2130: mol_type = other DNA
taatacgactcactataggggataaaaaaagttatcaggcatgcacctggtagctagtctttaaaccaatagattgcatcggtttaaaaggcaagaccgtcaaattgcgggaaaggggtcaacagccgttcagtaccaagtctcaggggaaactttgagatggccttgcaaagggtatggtaataagctgacggacatggtcctaaccacgcagccaagtcctaagtcaacagatcttctgttgatatggatgcagttcacagactaaatgtcggtcggggaagatgtattcttctcataagatatagtcggacctctccttaatgggagctagcggatgaagtgatgcaacactggagccgctgggaactaatttgtatgcgaaagtatattgattagttttggagtactcgcctatactggctgcttatggtgacaattgagagatcgttaccatatagctattggattggccatccggtgactaatagagctattatatatccctttgttgggtttataccacttagcttgaaagaggttaaaacattacaattcattgttaagttgaatacagcaaaatggcttccaaggtgtacgaccccgagcaacgcaaacgcatgatcactgggcctcagtggtgggctcgctgcaagcaaatgaacgtgctggactccttcatcaactactatgattccgagaagcacgccgagaacgccgtgatttttctgcatggtaacgctgcctccagctacctgtggaggcacgtcgtgcctcacatcgagcccgtggctagatgcatcatccctgatctgatcggaatgggtaagtccggcaagagcgggaatggctcatatcgcctcctggatcactacaagtacctcaccgcttggttcgagctgctgaaccttccaaagaaaatcatctttgtgggccacgactggggggcttgtctggcctttcactactcctacgagcaccaagacaagatcaaggccatcgtccatgctgagagtgtcgtggacgtgatcgagtcctgggacgagtggcctgacatcgaggaggatatcgccctgatcaagagcgaagagggcgagaaaatggtgcttgagaataacttcttcgtcgagaccgtcctcccaagcaagatcatgcggaaactggagcctgaggagttcgctgcctacctggagccattcaaggagaagggcgaggttagacggcctaccctctcctggcctcgcgagatccctctcgttaagggaggcaagcccgacgtcgtcgcaattgtccgcaactacaacgcctaccttcgggccagcgacgatctgcctaagatgttcatcgagtccgaccctgggttcttttccaacgctattgtcgagggagctaagaagttccctaacaccgagttcgtgaaggtgaagggcctccacttcagccaggaggacgctccagatgaaatgggtaagtacatcaagagcttcgtggagcgcgtgctgaagaacgagcagtaaaaaaaacaaaaaacaaaacaaaaacaaaaaacaaaaaaaattaaaacagcctgtgggttgatcccacccacaggcccattgggcgctagcactctggtatcacggtacctttgtgcgcctgttttataccccctcccccaactgtaacttagaagtaacacacaccgatcaacagtcagcgtggcacaccagccacgttttgatcaagcacttctgttaccccggactgagtatcaatagactgctcacgcggttgaaggagaaagcgttcgttatccggccaactacttcgaaaaacctagtaacaccgtggaagttgcagagtgtttcgctcagcactaccccagtgtagatcaggtcgatgagtcaccgcattccccacgggcgaccgtggcggtggctgcgttggcggcctgcccatggggaaacccatgggacgctctaatacagacatggtgcgaagagtctattgagctagttggtagtcctccggcccctgaatgcggctaatcctaactgcggagcacacaccctcaagccagagggcagtgtgtcgtaacgggcaactctgcagcggaaccgactactttgggtgtccgtgtttcattttatt

SEQ ID NO: 97 - DNA, 2502 bp, synthetic construct
  misc_feature 1..2502: note = Fig. 27a_GOI: CVB3 IRES-F.Luciferase
  source 1..2502: mol_type = other DNA
ttaaaacagcctgtgggttgatcccacccacaggcccattgggcgctagcactctggtatcacggtacctttgtgcgcctgttttataccccctcccccaactgtaacttagaagtaacacacaccgatcaacagtcagcgtggcacaccagccacgttttgatcaagcacttctgttaccccggactgagtatcaatagactgctcacgcggttgaaggagaaagcgttcgttatccggccaactacttcgaaaaacctagtaacaccgtggaagttgcagagtgtttcgctcagcactaccccagtgtagatcaggtcgatgagtcaccgcattccccacgggcgaccgtggcggtggctgcgttggcggcctgcccatggggaaacccatgggacgctctaatacagacatggtgcgaagagtctattgagctagttggtagtcctccggcccctgaatgcggctaatcctaactgcggagcacacaccctcaagccagagggcagtgtgtcgtaacgggcaactctgcagcggaaccgactactttgggtgtccgtgtttcattttattcctatactggctgcttatggtgacaattgagagatcgttaccatatagctattggattggccatccggtgactaatagagctattatatatccctttgttgggtttataccacttagcttgaaagaggttaaaacattacaattcattgttaagttgaatacagcaaaatggaagacgccaaaaacataaagaaaggcccggcgccattctatccgctggaagatggaaccgctggagagcaactgcataaggctatgaagagatacgccctggttcctggaacaattgcttttacagatgcacatatcgaggtggacatcacttacgctgagtacttcgaaatgtccgttcggttggcagaagctatgaaacgatatgggctgaatacaaatcacagaatcgtcgtatgcagtgaaaactctcttcaattctttatgccggtgttgggcgcgttatttatcggagttgcagttgcgcccgcgaacgacatttataatgaacgtgaattgctcaacagtatgggcatttcgcagcctaccgtggtgttcgtttccaaaaaggggttgcaaaaaattttgaacgtgcaaaaaaagctcccaatcatccaaaaaattattatcatggattctaaaacggattaccagggatttcagtcgatgtacacgttcgtcacatctcatctacctcccggttttaatgaatacgattttgtgccagagtccttcgatagggacaagacaattgcactgatcatgaactcctctggatctactggtctgcctaaaggtgtcgctctgcctcatagaactgcctgcgtgagattctcgcatgccagagatcctatttttggcaatcaaatcattccggatactgcgattttaagtgttgttccattccatcacggttttggaatgtttactacactcggatatttgatatgtggatttcgagtcgtcttaatgtatagatttgaagaagagctgtttctgaggagccttcaggattacaagattcaaagtgcgctgctggtgccaaccctattctccttcttcgccaaaagcactctgattgacaaatacgatttatctaatttacacgaaattgcttctggtggcgctcccctctctaaggaagtcggggaagcggttgccaagaggttccatctgccaggtatcaggcaaggatatgggctcactgagactacatcagctattctgattacacccgagggggatgataaaccgggcgcggtcggtaaagttgttccattttttgaagcgaaggttgtggatctggataccgggaaaacgctgggcgttaatcaaagaggcgaactgtgtgtgagaggtcctatgattatgtccggttatgtaaacaatccggaagcgaccaacgccttgattgacaaggatggatggctacattctggagacatagcttactgggacgaagacgaacacttcttcatcgttgaccgcctgaagtctctgattaagtacaaaggctatcaggtggctcccgctgaattggaatccatcttgctccaacaccccaacatcttcgacgcaggtgtcgcaggtcttcccgacgatgacgccggtgaacttcccgccgccgttgttgttttggagcacggaaagacgatgacggaaaaagagatcgtggattacgtcgccagtcaagtaacaaccgcgaaaaagttgcgcggaggagttgtgtttgtggacgaagtaccgaaaggtcttaccggaaaactcgacgcaagaaaaatcagagagatcctcataaaggccaagaagggcggaaagatcgccgtgtaaaaaaaacaaaaaacaaaacggctattatgcgttaccggcgccggaaacgcaatagccgaaaaacaaaaaacaaaaaaaacaaaaaaaaaaccaaaaaaacaaaacaca

SEQ ID NO: 98 - DNA, 2915 bp, synthetic construct
  misc_feature 1..2915: note = Fig. 27b_DNA template for expression of self-circularization RNA comprising recontructed GOI(CVB3 IRES-F.Luciferase)
  source 1..2915: mol_type = other DNA
taatacgactcactataggggataaaaaaagttatcaggcatgcacctggtagctagtctttaaaccaatagattgcatcggtttaaaaggcaagaccgtcaaattgcgggaaaggggtcaacagccgttcagtaccaagtctcaggggaaactttgagatggccttgcaaagggtatggtaataagctgacggacatggtcctaaccacgcagccaagtcctaagtcaacagatcttctgttgatatggatgcagttcacagactaaatgtcggtcggggaagatgtattcttctcataagatatagtcggacctctccttaatgggagctagcggatgaagtgatgcaacactggagccgctgggaactaatttgtatgcgaaagtatattgattagttttggagtactcgcctatactggctgcttatggtgacaattgagagatcgttaccatatagctattggattggccatccggtgactaatagagctattatatatccctttgttgggtttataccacttagcttgaaagaggttaaaacattacaattcattgttaagttgaatacagcaaaatggaagacgccaaaaacataaagaaaggcccggcgccattctatccgctggaagatggaaccgctggagagcaactgcataaggctatgaagagatacgccctggttcctggaacaattgcttttacagatgcacatatcgaggtggacatcacttacgctgagtacttcgaaatgtccgttcggttggcagaagctatgaaacgatatgggctgaatacaaatcacagaatcgtcgtatgcagtgaaaactctcttcaattctttatgccggtgttgggcgcgttatttatcggagttgcagttgcgcccgcgaacgacatttataatgaacgtgaattgctcaacagtatgggcatttcgcagcctaccgtggtgttcgtttccaaaaaggggttgcaaaaaattttgaacgtgcaaaaaaagctcccaatcatccaaaaaattattatcatggattctaaaacggattaccagggatttcagtcgatgtacacgttcgtcacatctcatctacctcccggttttaatgaatacgattttgtgccagagtccttcgatagggacaagacaattgcactgatcatgaactcctctggatctactggtctgcctaaaggtgtcgctctgcctcatagaactgcctgcgtgagattctcgcatgccagagatcctatttttggcaatcaaatcattccggatactgcgattttaagtgttgttccattccatcacggttttggaatgtttactacactcggatatttgatatgtggatttcgagtcgtcttaatgtatagatttgaagaagagctgtttctgaggagccttcaggattacaagattcaaagtgcgctgctggtgccaaccctattctccttcttcgccaaaagcactctgattgacaaatacgatttatctaatttacacgaaattgcttctggtggcgctcccctctctaaggaagtcggggaagcggttgccaagaggttccatctgccaggtatcaggcaaggatatgggctcactgagactacatcagctattctgattacacccgagggggatgataaaccgggcgcggtcggtaaagttgttccattttttgaagcgaaggttgtggatctggataccgggaaaacgctgggcgttaatcaaagaggcgaactgtgtgtgagaggtcctatgattatgtccggttatgtaaacaatccggaagcgaccaacgccttgattgacaaggatggatggctacattctggagacatagcttactgggacgaagacgaacacttcttcatcgttgaccgcctgaagtctctgattaagtacaaaggctatcaggtggctcccgctgaattggaatccatcttgctccaacaccccaacatcttcgacgcaggtgtcgcaggtcttcccgacgatgacgccggtgaacttcccgccgccgttgttgttttggagcacggaaagacgatgacggaaaaagagatcgtggattacgtcgccagtcaagtaacaaccgcgaaaaagttgcgcggaggagttgtgtttgtggacgaagtaccgaaaggtcttaccggaaaactcgacgcaagaaaaatcagagagatcctcataaaggccaagaagggcggaaagatcgccgtgtaaaaaaaacaaaaaacaaaacggctattatgcgttaccggcgccggaaacgcaatagccgaaaaacaaaaaacaaaaaaaacaaaaaaaaaaccaaaaaaacaaaacacattaaaacagcctgtgggttgatcccacccacaggcccattgggcgctagcactctggtatcacggtacctttgtgcgcctgttttataccccctcccccaactgtaacttagaagtaacacacaccgatcaacagtcagcgtggcacaccagccacgttttgatcaagcacttctgttaccccggactgagtatcaatagactgctcacgcggttgaaggagaaagcgttcgttatccggccaactacttcgaaaaacctagtaacaccgtggaagttgcagagtgtttcgctcagcactaccccagtgtagatcaggtcgatgagtcaccgcattccccacgggcgaccgtggcggtggctgcgttggcggcctgcccatggggaaacccatgggacgctctaatacagacatggtgcgaagagtctattgagctagttggtagtcctccggcccctgaatgcggctaatcctaactgcggagcacacaccctcaagccagagggcagtgtgtcgtaacgggcaactctgcagcggaaccgactactttgggtgtccgtgtttcattttatt